European Patent Application EP 4 310 503 A2, published January 24, 2024. Title: METHODS RELATED TO BIOLOGICS. Applicant: Momenta Pharmaceuticals, Inc. Application EP, filed December 28, 2016. The sequence listing filed with the application follows.

SEQUENCE LISTING (2 sequences)

SEQ ID NO: 1 - protein, 449 aa, synthetic construct
  REGION 1..449: note = Description of Artificial Sequence: Synthetic polypeptide
EVQLVQSGAEVKKPGESLKISCKGSGYSFTTYWLGWVRQMPGKGLDWIGIMSPVDSDIRYSPSFQGQVTMSVDKSITTAYLQWNSLKASDTAMYYCARRRPGQGYFDFWGQGTLVTVSSASTKGPSVFPLAPSSKSTSGGTAALGCLVKDYFPEPVTVSWNSGALTSGVHTFPAVLQSSGLYSLSSVVTVPSSSLGTQTYICNVNHKPSNTKVDKKVEPKSCDKTHTCPPCPAPELLGGPSVFLFPPKPKDTLMISRTPEVTCVVVDVSHEDPEVKFNWYVDGVEVHNAKTKPREEQYNSTYRVVSVLTVLHQDWLNGKEYKCKVSNKALPAPIEKTISKAKGQPREPQVYTLPPSRDELTKNQVSLTCLVKGFYPSDIAVEWESNGQPENNYKTTPPVLDSDGSFFLYSKLTVDKSRWQQGNVFSCSVMHEALHNHYTQKSLSLSPGK

SEQ ID NO: 2 - protein, 165 aa, synthetic construct
  REGION 1..165: note = Description of Artificial Sequence: Synthetic polypeptide
DIQMTQSPSSLSASVGDRVTITCRASQGISSWLAWYQQKPEKAPKSLIYAASSLQSGVPSRFSGSGSGTDFTLTISSLQEDFATYYCQQYNIYPYTFGQGTKLEIKRTVAAPSVFIFPPSDEQLKSGTASVVCLLNNFYPREAKVQWKVDNALQSGNSQESVTEQ